European Patent Specification EP 3 774 884 B1, published December 6, 2023. Title: METHODS OF GENERATING BROADLY PROTECTIVE VACCINE COMPOSITIONS COMPRISING HEMAGGLUTININ. Applicant: SANOFI PASTEUR INC. The sequence listing filed with the application follows.

SEQUENCE LISTING (33 sequences)

SEQ ID NO: 1 - protein, 566 aa, Artificial Sequence
  source: /note="Description of Artificial Sequence: Synthetic polypeptide"
MKAILVVLLYTFATANADTLCIGYHANNSTDTVDTVLEKNVTVTHSVNLLEDKHNGKLCKLRGVAPLHLGKCNIAGWILGNPECESLSTASSWSYIVETSSSDNGTCYPGDFIDYEELREQLSSVSSFERFEIFPKTSSWPNHDSNKGVTAACPHAGAKSFYKNLIWLVKKGNSYPKLSKSYINDKGKEVLVLWGIHHPSTSADQQSLYQNADAYVFVGTSRYSKKFKPEIAIRPKVRDQEGRMNYYWTLVEPGDKITFEATGNLVVPRYAFAMERNAGSGIIISDTPVHDCNTTCQTPKGAINTSLPFQNIHPITIGKCPKYVKSTKLRLATGLRNVPSIQSRGLFGAIAGFIEGGWTGMVDGWYGYHHQNEQGSGYAADLKSTQNAIDEITNKVNSVIEKMNTQFTAVGKEFNHLEKRIENLNKKVDDGFLDIWTYNAELLVLLENERTLDYHDSNVKNLYEKVRSQLKNNAKEIGNGCFEFYHKCDNTCMESVKNGTYDYPKYSEEAKLNREEIDGVKLESTRIYQILAIYSTVASSLVLVVSLGAISFWMCSNGSLQCRICI

SEQ ID NO: 2 - protein, 566 aa, Artificial Sequence
  source: /note="Description of Artificial Sequence: Synthetic polypeptide"
MKAILVVLLYTFATANADTLCIGYHANNSTDTVDTVLEKNVTVTHSVNLLEDRHNGKLCKLRGVAPLHLGKCNIAGWLLGNPECELLFTASSWSYIVETSNSDNGTCYPGDFINYEELREQLSSVSSFERFEIFPKASSWPNHETNRGVTAACPYAGANSFYRNLIWLVKKGNSYPKLSKSYVNNKGKEVLVLWGIHHPPTSTDQQSLYQNADAYVFVGSSKYNKKFKPEIATRPKVRGQAGRMNYYWTLIEPGDTITFEATGNLVVPRYAFAMKRGSGSGIIISDAPVHDCNTTCQTPKGAINTSLPFQNIHPVTIGECPKYVKSTKLRMATGLRNIPSIQSRGLFGAIAGFIEGGWTGMIDGWYGYHHQNEQGSGYAADQKSTQNAIDGITNKVNSVIEKMNTQFTAVGKEFNHLEKRIENLNKKVDDGFLDIWTYNAELLVLLENERTLDYHDSNVKNLYEKVRSQLKNNAKEIGNGCFEFYHKCDDTCMESVKNGTYDYPKYSEESKLNREKIDGVKLESMGVYQILAIYSTVASSLVLLVSLGAISFWMCSNGSLQCRICI

SEQ ID NO: 3 - protein, 565 aa, Artificial Sequence
  source: /note="Description of Artificial Sequence: Synthetic polypeptide"
MKVKLLVLLCTFTATYADTICIGYHANNSTDTVDTVLEKNVTVTHSVNLLENSHNGKLCLLKGIAPLQLGNCSVAGWILGNPECELLISKESWSYIVEKPNPENGTCYPGHFADYEELREQLSSVSSFERFEIFPKESSWPNHTVTGVSASCSHNGESSFYRNLLWLTGKNGLYPNLSKSYANNKEKEVLVLWGVHHPPNIGDQKTLYHTENAYVSVVSSHYSRKFTPEIAKRPKVRDQEGRINYYWTLLEPGDTIIFEANGNLIAPRYAFALSRGFGSGIINSNAPMDKCDAKCQTPQGAINSSLPFQNVHPVTIGECPKYVRSAKLRMVTGLRNIPSIQSRGLFGAIAGFIEGGWTGMVDGWYGYHHQNEQGSGYAADQKSTQNAINGITNKVNSVIEKMNTQFTAVGKEFNKLERRMENLNKKVDDGFIDIWTYNAELLVLLENERTLDFHDSNVKNLYEKVKSQLKNNAKEIGNGCFEFYHKCNDECMESVKNGTYDYPKYSEESKLNREKIDGVKLESMGVYQILAIYSTVASSLVLLVSLGAISFWMCSNGSLQCRICI

SEQ ID NO: 4 - protein, 565 aa, Artificial Sequence
  source: /note="Description of Artificial Sequence: Synthetic polypeptide"
MKVKLLVLLCTFTATYADTICIGYHANNSTDTVDTVLEKNVTVTHSVNLLEDSHNGKLCLLKGIAPLQLGNCSVAGWILGNPECELLISKESWSYIVETPNPENGTCYPGYFADYEELREQLSSVSSFERFEIFPKESSWPNHTVTGVSASCSHNGKSSFYRNLLWLTGKNGLYPNLSKSYANNKEKEVLVLWGVHHPPNIGDQRALYHTENAYVSVVSSHYSRRFTPEIAKRPKVRDQEGRINYYWTLLEPGDTIIFEANGNLIAPRFAFALSRGFGSGIITSNAPMDECDAKCQTPQGAINSSLPFQNVHPVTIGECPKYVRSAKLRMVTGLRNIPSIQSRGLFGAIAGFIEGGWTGMVDGWYGYHHQNEQGSGYAADQKSTQNAINGITNKVNSVIEKMNTQFTAVGKEFNKLERRMENLNKKVDDGFLDIWTYNAELLVLLENERTLDFHDSNVKNLYEKVKSQLKNNAKEIGNGCFEFYHKCNDECMESVKNGTYDYPKYSEESKLNRERIDGVKLESMGVYQILAIYSTVASSLVLLVSLGAISFWMCSNGSLQCRICI

SEQ ID NO: 5 - protein, 566 aa, Artificial Sequence
  source: /note="Description of Artificial Sequence: Synthetic polypeptide"
MKVKLLVLLCAFTATYADTICIGYHANNSTDTVDTVLEKNVTVTHSVNLLEDSHNGKLCRLKGTAPLQLGNCSVAGWILGNPECESLFSKESWSYIAETPNPENGTCYPGYFADYEELREQLSSVSSFERFEIFPKESSWPNHTVTKGVTASCSHNGKSSFYKNLLWLTEKNGLYPNLSKSYVNNKEKEVLVLWGVHHPSNIGDQRAIYHTENAYVSVVSSHYSRRFTPEIAKRPKVRDQEGRINYYWTLLEPGDTIIFEANGNLIAPWYAFALSRGFGSGIITSNASMGECDAKCQTPQGAINSSLPFQNVHPVTIGECPKYVRSTKLRMVTGLRNIPSIQSRGLFGAIAGFIEGGWTGMIDGWYGYHHQNEQGSGYAADQKSTQNAIDGITNKVNSVIEKMNTQFTAVGKEFNKLERRMENLNKKVDDGFLDIWTYNAELLVLLENERTLDFHDSNVKNLYEKVKNQLKNNAKEIGNGCFEFYHKCNNECMESVKNGTYDYPKYSEESKLNREKIDGVKLESMGVYQILAIYSTVASSLVLLVSLGAISFWMCSNGSLQCRICI

SEQ ID NO: 6 - protein, 566 aa, Artificial Sequence
  source: /note="Description of Artificial Sequence: Synthetic polypeptide"
MKAKLLVLLCTFTATYADTICIGYHANNSTDTVDTVLEKNVTVTHSVNLLEDSHNGKLCRLKGIAPLQLGKCSIAGWILGNPECESLFSKKSWSYIAETPNSENGTCYPGYFADYEELREQLSSVSSFERFEIFPKERSWPKHNVTRGVTASCSHKGKSSFYRNLLWLTEKNGSYPNLSKSYVNNKEKEVLVLWGVHHPSNIEDQKTIYRKENAYVSVVSSNYNRRFTPEIAKRPKVRGQEGRINYYWTLLEPGDTIIFEANGNLIAPWYAFALSRGFGSGIITSNASMDECDAKCQTPQGAINSSLPFQNVHPVTIGECPKYVRSTKLRMVTGLRNIPSIQSRGLFGAIAGFIEGGWTGMIDGWYGYHHQNEQGSGYAADQKSTQNAINGITNKVNSVIEKMNTQFTAVGKEFNKLEKRMENLNKKVDDGFLDIWTYNAELLVLLENERTLDFHDSNVKNLYEKVKSQLKNNAKEIGNGCFEFYHKCNNECMESVKNGTYDYPKYSEESKLNREKIDGVKLESMGVYQILAIYSTVASSLVLLVSLGAISFWMCSNGSLQCRICI

SEQ ID NO: 7 - protein, 566 aa, Artificial Sequence
  source: /note="Description of Artificial Sequence: Synthetic polypeptide"
MKAKLLVLLCTFTATYADTICIGYHANNSTDTVDTVLEKNVTVTHSVNLLEDSHNGKLCRLKGIAPLQLGKCNIAGWILGNPECESLLSNRSWSYIAETPNSENGTCYPGDFADYEELREQLSSVSSFERFEIFPKERSWPKHNTTRGVTAACSHAKKSSFYKNLLWLTEKNGSYPNLSRSYVNNKEKEVLVLWGVHHPSNIEDQRTLYRKENAYVSVVSSNYNRRFTPEIAERPKVRGQAGRMNYYWTLLEPGDTIIFEANGNLIAPWYAFALSRGLGSGIITSNASMDECDTKCQTPQGAINSSLPFQNIHPVTIGECPKYVRSTKLRMVTGLRNIPSIQSRGLFGAIAGFIEGGWTGMMDGWYGYHHQNEQGSGYAADQKSTQNAINGITNKVNSVIEKMNTQFTAVGKEFNKLEKRMENLNKKVDDGFLDIWTYNAELLVLLENERTLDFHDSNVKNLYEKVKNQLRNNAKEIGNGCFEFYHKCDNECMESVKNGTYDYPKYSEESKLNREKIDGVKLESMGVYQILAIYSTVASSLVLLVSLGAISFWMCSNGSLQCRICI

SEQ ID NO: 8 - protein, 566 aa, Artificial Sequence
  source: /note="Description of Artificial Sequence: Synthetic polypeptide"
MKAKLLVLLCTFTATYADTICIGYHANNSTDTVDTVLEKNVTVTHSVNLLEDSHNGKLCRLKGIAPLQLGKCNIAGWLLGNPECDSLLPARSWSYIVETPNSENGICYPGDFIDYEELREQLSSVSSFERFEIFPKESSWPNHNTTNGVTAACSHEGKSSFYRNLLWLTKKEGSYPKLKNSYVNKKGKEVLVLWGVHHPSNSKEQQNLYQNENAYVSVVSSNYNRRFTPEIAERPKVRDQAGRMNYYWTLLKPGDTIIFEANGNLIAPWYAFALSRGFGSGIITSNASMHECNTKCQTPLGAINSSLPFQNIHPVTIGECPKYVRSAKLRMVTGLRNIPSIQSRGLFGAIAGFIEGGWTGMIDGWYGYHHQNEQGSGYAADQKSTQNAINGITNKVNSVIEKMNTQFTAVGKEFNNLEKRMENLNKKVDDGFLDIWTYNAELLVLLENERTLDFHDSNVKNLYEKVKSQLKNNAKEIGNGCFEFYHKCDNECMESVRNGTYDYPKYSEESKLNREKIDGVKLESMGVYQILAIYSTVASSLVLLVSLGAISFWMCSNGSLQCRICI

SEQ ID NO: 9 - protein, 566 aa, Artificial Sequence
  source: /note="Description of Artificial Sequence: Synthetic polypeptide"
MKAILVVLLYTFATANADTLCIGYHANNSTDTVDTVLEKNVTVTHSVNLLEDKHNGKLCKLRGVAPLHLGKCNIAGWILGNPECESLFTASSWSYIVETSNSDNGTCYPGDFINYEELREQLSSVSSFERFEIFPKTSSWPNHDTNRGVTAACPHAGAKSFYRNLIWLVKKGNSYPKLSKSYINDKGKEVLVLWGIHHPSTSADQQSLYQNADAYVFVGSSKYSKKFKPEIATRPKVRDQAGRMNYYWTLVEPGDTITFEATGNLVVPRYAFAMKRGSGSGIIISDTPVHDCNTTCQTPKGAINTSLPFQNIHPVTIGECPKYVKSTKLRMATGLRNVPSIQSRGLFGAIAGFIEGGWTGMVDGWYGYHHQNEQGSGYAADQKSTQNAIDGITNKVNSVIEKMNTQFTAVGKEFNHLEKRIENLNKKVDDGFLDIWTYNAELLVLLENERTLDYHDSNVKNLYEKVRSQLKNNAKEIGNGCFEFYHKCDNTCMESVKNGTYDYPKYSEEAKLNREEIDGVKLESTRIYQILAIYSTVASSLVLVVSLGAISFWMCSNGSLQCRICI

SEQ ID NO: 10 - protein, 566 aa, Artificial Sequence
  source: /note="Description of Artificial Sequence: Synthetic polypeptide"
MKAKLLVLLCALSATDADTICIGYHANNSTDTVDTVLEKNVTVTHSVNLLEDSHNGKLCRLKGIAPLQLGKCSIAGWILGNPECESLFSKKSWSYIAETPNSENGTCYPGYFADYEELREQLSSVSSFERFEIFPKERSWPKHNITRGVTAACSHKGKSSFYRNLLWLTEKNGSYPNLSKSYVNNKEKEVLVLWGVHHPSNIEDQKTLYRKENAYVSVVSSNYNRRFTPEIAKRPKVRGQEGRINYYWTLLEPGDTIIFEANGNLIAPWYAFALSRGFGSGIITSNASMDECDTKCQTPQGAINSSLPFQNVHPVTIGECPKYVRSTKLRMVTGLRNIPSIQSRGLFGAIAGFIEGGWTGMIDGWYGYHHQNEQGSGYAADQKSTQNAINGITNKVNSVIEKMNTQFTAVGKEFNKLEKRMENLNKKVDDGFLDIWTYNAELLVLLENERTLDFHDSNVKNLYEKVKNQLKNNAKEIGNGCFEFYHKCNNECMESVKNGTYDYPKYSEESKLNREKIDGVKLESMGVYQILAIYSTVASSLVLLVSLGAISFWMCSNGSLQCRICI

SEQ ID NO: 11 - protein, 565 aa, Artificial Sequence
  source: /note="Description of Artificial Sequence: Synthetic polypeptide"
MKVKLLVLLCTFTATYADTICIGYHANNSTDTVDTVLEKNVTVTHSVNLLEDSHNGKLCLLKGIAPLQLGNCSVAGWILGNPECELLISKESWSYIVETPNPENGTCYPGYFADYEELREQLSSVSSFERFEIFPKESSWPNHTVTGVSASCSHNGKSSFYRNLLWLTGKNGLYPNLSKSYTNNKEKEVLVLWGVHHPPNIGDQRALYHTENAYVSVVSSHYSRRFTPEIAKRPKVRDQEGRINYYWTLLEPGDTIIFEANGNLIAPRYAFALSRGFGSGIITSNAPMDECDAKCQTPQGAINSSLPFQNVHPVTIGECPKYVRSAKLRMVTGLRNIPSIQSRGLFGAIAGFIEGGWTGMVDGWYGYHHQNEQGSGYAADQKSTQNAINGITNKVNSVIEKMNTQFTAVGKEFNKLERRMENLNKKVDDGFLDIWTYNAELLVLLENERTLDFHDSNVKNLYEKVKSQLKNNAKEIGNGCFEFYHKCNDECMESVKNGTYDYPKYSEESKLNREKIDGVKLESMGVYQILAIYSTVASSLVLLVSLGAISFWMCSNGSLQCRICI

SEQ ID NO: 12 - protein, 566 aa, Artificial Sequence
  source: /note="Description of Artificial Sequence: Synthetic polypeptide"
MKAKLLVLLCTFTATYADTICIGYHANNSTDTVDTVLEKNVTVTHSVNLLEDSHNGKLCRLKGIAPLQLGKCNIAGWILGNPECESLFSKESWSYIVETPNSENGTCYPGDFADYEELREQLSSVSSFERFEIFPKESSWPNHNTTRGVTAACSHNGKSSFYRNLLWLTKKNGSYPNLSKSYVNNKEKEVLVLWGVHHPSNIGDQQTLYQNENAYVSVVSSNYSRRFTPEIAKRPKVRDQEGRMNYYWTLLEPGDTIIFEANGNLIAPRYAFALSRGFGSGIITSNASMDECDTKCQTPQGAINSSLPFQNIHPVTIGECPKYVRSTKLRMVTGLRNIPSIQSRGLFGAIAGFIEGGWTGMIDGWYGYHHQNEQGSGYAADQKSTQNAINGITNKVNSVIEKMNTQFTAVGKEFNKLEKRMENLNKKVDDGFLDIWTYNAELLVLLENERTLDFHDSNVKNLYEKVKSQLKNNAKEIGNGCFEFYHKCDNECMESVKNGTYDYPKYSEEAKLNREEIDGVKLESMGVYQILAIYSTVASSLVLLVSLGAISFWMCSNGSLQCRICI

SEQ ID NO: 13 - protein, 566 aa, Artificial Sequence
  source: /note="Description of Artificial Sequence: Synthetic polypeptide"
MKAKLLVLLCTFTATYADTICIGYHANNSTDTVDTVLEKNVTVTHSVNLLEDSHNGKLCRLKGIAPLQLGKCNIAGWILGNPECESLFSKESWSYIVETPNSENGTCYPGDFADYEELREQLSSVSSFERFEIFPKESSWPNHNTTRGVTAACSHNGKSSFYRNLLWLTKKNGSYPNLSKSYVNNKEKEVLVLWGVHHPSNIGDQQTLYQNENAYVSVVSSNYSRRFTPEIAKRPKVRDQEGRMNYYWTLLEPGDTIIFEANGNLIAPRYAFALSRGFGSGIITSNAPMDECDTKCQTPQGAINSSLPFQNIHPVTIGECPKYVRSTKLRMVTGLRNIPSIQSRGLFGAIAGFIEGGWTGMIDGWYGYHHQNEQGSGYAADQKSTQNAINGITNKVNSVIEKMNTQFTAVGKEFNKLEKRMENLNKKVDDGFLDIWTYNAELLVLLENERTLDFHDSNVKNLYEKVKSQLKNNAKEIGNGCFEFYHKCDNECMESVKNGTYDYPKYSEEAKLNREEIDGVKLESMGVYQILAIYSTVASSLVLLVSLGAISFWMCSNGSLQCRICI

SEQ ID NO: 14 - protein, 566 aa, Artificial Sequence
  source: /note="Description of Artificial Sequence: Synthetic polypeptide"
MKAKLLVLLCTFTATYADTICIGYHANNSTDTVDTVLEKNVTVTHSVNLLEDSHNGKLCRLKGIAPLQLGKCNIAGWILGNPECESLFSKESWSYIVETPNSENGTCYPGDFADYEELREQLSSVSSFERFEIFPKESSWPNHNTTRGVTAACSHNGKSSFYRNLLWLTKKNGSYPNLSKSYVNNKEKEVLVLWGVHHPSNIGDQQTLYQNENAYVSVVSSNYSRRFTPEIAKRPKVRDQEGRMNYYWTLLEPGDTIIFEANGNLIAPWYAFALSRGFGSGIITSNASMDECDTKCQTPQGAINSSLPFQNIHPVTIGECPKYVRSTKLRMVTGLRNIPSIQSRGLFGAIAGFIEGGWTGMIDGWYGYHHQNEQGSGYAADQKSTQNAINGITNKVNSVIEKMNTQFTAVGKEFNKLEKRMENLNKKVDDGFLDIWTYNAELLVLLENERTLDFHDSNVKNLYEKVKSQLKNNAKEIGNGCFEFYHKCDNECMESVKNGTYDYPKYSEEAKLNREEIDGVKLESMGVYQILAIYSTVASSLVLLVSLGAISFWMCSNGSLQCRICI

SEQ ID NO: 15 - protein, 566 aa, Artificial Sequence
  source: /note="Description of Artificial Sequence: Synthetic polypeptide"
MKAKLLVLLCTFTATYADTICIGYHANNSTDTVDTVLEKNVTVTHSVNLLEDSHNGKLCRLKGIAPLQLGKCNIAGWILGNPECESLFSKESWSYIVETPNSENGTCYPGDFADYEELREQLSSVSSFERFEIFPKESSWPNHNVTRGVTAACSHNGKSSFYRNLLWLTKKNGSYPNLSKSYVNNKEKEVLVLWGVHHPSNIGDQQTLYQNENAYVSVVSSNYSRRFTPEIAKRPKVRDQEGRMNYYWTLLEPGDTIIFEANGNLIAPRYAFALSRGFGSGIITSNASMDECDTKCQTPQGAINSSLPFQNIHPVTIGECPKYVRSTKLRMVTGLRNIPSIQSRGLFGAIAGFIEGGWTGMIDGWYGYHHQNEQGSGYAADQKSTQNAINGITNKVNSVIEKMNTQFTAVGKEFNKLEKRMENLNKKVDDGFLDIWTYNAELLVLLENERTLDFHDSNVKNLYEKVKSQLKNNAKEIGNGCFEFYHKCDNECMESVKNGTYDYPKYSEEAKLNREEIDGVKLESMGVYQILAIYSTVASSLVLLVSLGAISFWMCSNGSLQCRICI

SEQ ID NO: 16 - protein, 566 aa, Artificial Sequence
  source: /note="Description of Artificial Sequence: Synthetic polypeptide"
MKAKLLVLLCTFTATYADTICIGYHANNSTDTVDTVLEKNVTVTHSVNLLEDSHNGKLCRLKGIAPLQLGKCNIAGWILGNPECESLFSKESWSYIVETPNSENGTCYPGDFADYEELREQLSSVSSFERFEIFPKESSWPNHNVTRGVTAACSHNGKSSFYRNLLWLTKKNGSYPNLSKSYVNNKEKEVLVLWGVHHPSNIGDQQTLYQNENAYVSVVSSNYSRRFTPEIAKRPKVRDQEGRMNYYWTLLEPGDTIIFEANGNLIAPWYAFALSRGFGSGIITSNASMDECDTKCQTPQGAINSSLPFQNIHPVTIGECPKYVRSTKLRMVTGLRNIPSIQSRGLFGAIAGFIEGGWTGMIDGWYGYHHQNEQGSGYAADQKSTQNAINGITNKVNSVIEKMNTQFTAVGKEFNKLEKRMENLNKKVDDGFLDIWTYNAELLVLLENERTLDFHDSNVKNLYEKVKSQLKNNAKEIGNGCFEFYHKCDNECMESVKNGTYDYPKYSEEAKLNREEIDGVKLESMGVYQILAIYSTVASSLVLLVSLGAISFWMCSNGSLQCRICI

SEQ ID NO: 17 - protein, 23 aa, Artificial Sequence
  source: /note="Description of Artificial Sequence: Synthetic peptide"
MPMGSLQPLATLYLLGMLVASVL

SEQ ID NO: 18 - protein, 8 aa, Artificial Sequence
  source: /note="Description of Artificial Sequence: Synthetic peptide"
WSHPQFEK

SEQ ID NO: 19 - protein, 40 aa, Artificial Sequence
  source: /note="Description of Artificial Sequence: Synthetic polypeptide"
  SITE (1)..(40): /note="This sequence may encompass 1-8 'Gly Gly Gly Gly Ser' repeating units"
GGGGSGGGGSGGGGSGGGGSGGGGSGGGGSGGGGSGGGGS

SEQ ID NO: 20 - protein, 16 aa, Artificial Sequence
  source: /note="Description of Artificial Sequence: Synthetic peptide"
GGSGGSGGGGSGGGGS

SEQ ID NO: 21 - protein, 5 aa, Artificial Sequence
  source: /note="Description of Artificial Sequence: Synthetic peptide"
GGGGS

SEQ ID NO: 22 - protein, 20 aa, Artificial Sequence
  source: /note="Description of Artificial Sequence: Synthetic peptide"
  SITE (1)..(20): /note="This sequence may encompass 1-4 'Gly Gly Gly Gly Ser' repeating units"
GGGGSGGGGSGGGGSGGGGS

SEQ ID NO: 23 - protein, 8 aa, Artificial Sequence
  source: /note="Description of Artificial Sequence: Synthetic peptide"
GGGGGGGG

SEQ ID NO: 24 - protein, 6 aa, Artificial Sequence
  source: /note="Description of Artificial Sequence: Synthetic peptide"
GGGGGG

SEQ ID NO: 25 - protein, 15 aa, Artificial Sequence
  source: /note="Description of Artificial Sequence: Synthetic peptide"
  SITE (1)..(15): /note="This sequence may encompass 1-3 'Glu Ala Ala Ala Lys' repeating units"
EAAAKEAAAKEAAAK

SEQ ID NO: 26 - protein, 27 aa, Artificial Sequence
  source: /note="Description of Artificial Sequence: Synthetic peptide"
  SITE (2)..(26): /note="This region may encompass 2-5 'Glu Ala Ala Ala Lys' repeating units"
AEAAAKEAAAKEAAAKEAAAKEAAAKA

SEQ ID NO: 27 - protein, 12 aa, Artificial Sequence
  source: /note="Description of Artificial Sequence: Synthetic peptide"
AEAAAKEAAAKA

SEQ ID NO: 28 - protein, 46 aa, Artificial Sequence
  source: /note="Description of Artificial Sequence: Synthetic polypeptide"
AEAAAKEAAAKEAAAKEAAAKALEAEAAAKEAAAKEAAAKEAAAKA

SEQ ID NO: 29 - protein, 5 aa, Artificial Sequence
  source: /note="Description of Artificial Sequence: Synthetic peptide"
PAPAP

SEQ ID NO: 30 - protein, 18 aa, Artificial Sequence
  source: /note="Description of Artificial Sequence: Synthetic peptide"
KESGSVSSEQLAQFRSLD

SEQ ID NO: 31 - protein, 14 aa, Artificial Sequence
  source: /note="Description of Artificial Sequence: Synthetic peptide"
EGKSSGSGSESKST

SEQ ID NO: 32 - protein, 12 aa, Artificial Sequence
  source: /note="Description of Artificial Sequence: Synthetic peptide"
GSAGSAAGSGEF

SEQ ID NO: 33 - protein, 6 aa, Artificial Sequence
  source: /note="Description of Artificial Sequence: Synthetic 6xHis tag"
HHHHHH